European Patent Application EP 4 545 549 A1, published April 30, 2025. Title: INSECT NEUROPEPTIDES 1. Applicant: SOLASTA Bio Limited. The sequence listing filed with the application follows.

SEQUENCE LISTING (16 sequences)

SEQ ID NO: 1 - protein, 12 aa, synthetic construct
  source 1..12: note = Z peptide
SPPYSPPFSPRL

SEQ ID NO: 2 - protein, 12 aa, synthetic construct
  source 1..12: note = SB-P-46
  MOD_RES 12: note = leucinamide
SPPYSPPFSPRL

SEQ ID NO: 3 - protein, 11 aa, synthetic construct
  source 1..11: note = SB-P-47
  MOD_RES 11: note = leucinamide
  MOD_RES 1: note = pyroglutamyl-alanine
AIMARPQVPRL

SEQ ID NO: 4 - protein, 8 aa, synthetic construct
  source 1..8: note = SB-P-49
  MOD_RES 8: note = leucinamide
SVPFKPRL

SEQ ID NO: 5 - protein, 19 aa, synthetic construct
  source 1..19: note = SB-P-51
  MOD_RES 19: note = leucinamide
LRQLQSNGEPAYRVRTPRL

SEQ ID NO: 6 - protein, 16 aa, synthetic construct
  source 1..16: note = SB-P-80
  MOD_RES 16: note = leucinamide
NADEDQQQSVDFTPRL

SEQ ID NO: 7 - protein, 10 aa, synthetic construct
  source 1..10: note = SB-P-81
  MOD_RES 10: note = leucinamide
GGSMTFSPRL

SEQ ID NO: 8 - protein, 8 aa, synthetic construct
  source 1..8: note = SB-P-70
  MOD_RES 8: note = glycinamide
KVKFSAWG

SEQ ID NO: 9 - protein, 10 aa, synthetic construct
  source 1..10: note = SB-P-65
  MOD_RES 10: note = glycinamide
RQKTVFSSWG

SEQ ID NO: 10 - protein, 7 aa, synthetic construct
  source 1..7: note = SB-P-66
  MOD_RES 7: note = glycinamide
PAFSSWG

SEQ ID NO: 11 - protein, 9 aa, synthetic construct
  source 1..9: note = SB-P-86
  MOD_RES 9: note = glycinamide
  MOD_RES 1: note = pyroglutamyl-leucine
LTFTSSWGG

SEQ ID NO: 12 - protein, 8 aa, synthetic construct
  source 1..8: note = SB-P-039
  MOD_RES 1: note = palmitoyl-glutamine
  MOD_RES 8: note = tryptophanamide
QLTFSPDW

SEQ ID NO: 13 - protein, 7 aa, synthetic construct
  source 1..7: note = SB-P-042
  MOD_RES 1: note = pyroglutamyl-leucine
  MOD_RES 7: note = tryptophanamide
LTFSPDW

SEQ ID NO: 14 - protein, 6 aa, synthetic construct
  source 1..6: note = SB-P-69
  MOD_RES 6: note = glycinamide
NFSPWG

SEQ ID NO: 15 - protein, 19 aa, synthetic construct
  source 1..19: note = SB-P-48
  MOD_RES 19: note = leucinamide
EQNVQSNGEPAYRVRTPRL

SEQ ID NO: 16 - protein, 8 aa, synthetic construct
  source 1..8: note = SB-P-41
  MOD_RES 8: note = tryptophanamide
QLTFSPDW